European Patent Specification EP 4 091 836 B1, published February 21, 2024. Title: PASSENGER CAR TIRE RUBBER COMPOSITION AND PASSENGER CAR TIRE. Applicant: SUMITOMO RUBBER INDUSTRIES,LTD. The sequence listing filed with the application follows.

SEQUENCE LISTING (10 sequences)

SEQ ID NO: 1 - DNA, 36 bp, Artificial Sequence
  Upstream primer（encP-U-Nde）
cgtacatatgatgaccttcgtcatagagctcgacat

SEQ ID NO: 2 - DNA, 26 bp, Artificial Sequence
  Downstream primer（encP-L-Bam）
tattggatcctcagtgcgccgccacg

SEQ ID NO: 3 - DNA, 21 bp, Artificial Sequence
  Upstream primer（FDC1-gU）
tcacgaaagtccaaattgcgt

SEQ ID NO: 4 - DNA, 21 bp, Artificial Sequence
  Downstream primer（FDC1-gL）
gttaatggcgcactgcttgtc

SEQ ID NO: 5 - DNA, 33 bp, Artificial Sequence
  Upstream primer（FDC1-nU-BspHI）
cgactcatgaggaagctaaatccagctttagaa

SEQ ID NO: 6 - DNA, 45 bp, Artificial Sequence
  Downstream primer（FDC1-nL-Hind）
gccaagcttatttatatccgtaccttttccaattttcatttactt

SEQ ID NO: 7 - DNA, 20 bp, Artificial Sequence
  Upstream primer（PAD1-gU）
gcattcctgtctgaaagcct

SEQ ID NO: 8 - DNA, 21 bp, Artificial Sequence
  Downstream primer（PAD1-gL）
tgatatcgggaagttcacggt

SEQ ID NO: 9 - DNA, 39 bp, Artificial Sequence
  Upstream primer（PAD1-nU-Nde）
cgtccatatgctcctatttccaagaagaactaatatagc

SEQ ID NO: 10 - DNA, 36 bp, Artificial Sequence
  Downstream primer（PAD1-nL－Xho）
cagtctcgagttacttgctttttattccttcccaac